European Patent Application EP 4 799 657 A1, published September 2, 2026. Title: IMPLANTABLE RECOMBINANT COLLAGEN MICROPARTICLE AND PREPARATION METHOD THEREFOR. Applicant: WitKang Zhiyuan Medical Devices (Xi'an) Co., Ltd. Application EP. The sequence listing filed with the application follows.

SEQUENCE LISTING (1 sequence)

SEQ ID NO: 1 - protein, 411 aa, Artificial Sequence
GPPGEPGNPGKPGSPGPAGSNGEPGPAGSPGEKGSQGSNGNPGPAGNQGQPGNKGSPGNPGKPGEPGSNGPQGEPGSQGNPGKNGQPGSPGSQGSPGNQGQPGKPGQPGEQGSPGNQGPAGNEGPKGQPGQNGKPGSPGPPGEPGNPGKPGSPGPAGSNGEPGPAGSPGEKGSQGSNGNPGPAGNQGQPGNKGSPGNPGKPGEPGSNGPQGEPGSQGNPGKNGQPGSPGSQGSPGNQGQPGKPGQPGEQGSPGNQGPAGNEGPKGQPGQNGKPGTPGPPGEPGNPGKPGSPGPAGSNGEPGPAGSPGEKGSQGSNGNPGPAGNQGQPGNKGSPGNPGKPGEPGSNGPQGEPGSQGNPGKNGQPGSPGSQGSPGNQGQPGKPGQPGEQGSPGNQGPAGNEGPKGQPGQNGKP